European Patent Application EP 4 800 030 A1, published September 2, 2026. Title: 一种识别EB病毒gB蛋白的单克隆抗体Fab5及其应用. Applicant: 中山大学肿瘤防治中心（中山大学附属肿瘤医院、中山大学肿瘤研究所）. Application WO. The sequence listing filed with the application follows.

SEQUENCE LISTING (25 sequences)

SEQ ID NO: 1 - protein, 691 aa, synthetic construct
MPMGSLQPLATLYLLGMLVASCLGQTPEQPAPPATTVQPTATRQQTSFPFRVCELSSHGDLFRFSSDIQCPSFGTRENHTEGLLMVFKDNIIPYSFKVRSYTKIVTNILIYNGHRADSVTNRHEEKFSVESYETDQMDTIYQCYNAVKMTKDGLTRVYVDRDGVNITVNLKPTGGLANGVRRYASQTELYDAPGRVEATYRTRTTVNCLITDMMAKSNSPFDFFVTTTGQTVEMSPFYDGKNTETFHERADSFHVRTNYKIVDYDNRGTNPQGERRAFLDKGTYTLSWKLENRTAYCPLQHWQTFDSTIATETGKSIHFVTDEGTSSFVTNTTVGIELPDAFKCIEEQVNKTMHEKYEAVQDRYTKGQEAITYFITSGGLLLAWLPLTPRSLATVKNLTELTTPTSSPPSSPSPPAPPAARGSTSAAVLRRRRRNAGNATTPVPPAAPGKSLGTLNNPATVQIQFAYDSLRRQINRMLGDLARAWCLEQKRQNMVLRELTKINPTTVMSSIYGKAVAAKRLGDVISVSQCVPVNQATVTLRKSMRVPGSETMCYSRPLVSFSFINDTKTYEGQLGTDNEIFLTKKMTEVCQATSQYYFQSGNEIHVYNDYHHFKTIELDGIATLQTFISLNTSLIENIDFASLELYSRDEQRASNVFDLEGIFREYNFQAQNIAGLRKDLDNAVSHHHHHH

SEQ ID NO: 2 - DNA, 2073 bp, synthetic construct
  source 1..2073: mol_type = other DNA
atgccaatgggctctctgcagcccctggccacactgtacctgctgggaatgctggtggcaagctgcctgggacagaccccagagcagcctgcaccacctgccaccacagtgcagcctacagccaccagacagcagaccagcttccccttccgggtgtgcgagctgagctcccacggcgacctgttcagattttctagcgatatccagtgtccctccttcggcacaagggagaaccacaccgagggcctgctgatggtgttcaaggacaatatcatcccttactcctttaaggtgagatcttatacaaagatcgtgaccaacatcctgatctacaatggccacagagccgattctgtgaccaacaggcacgaggagaagtttagcgtggagtcctatgagacagaccagatggataccatctaccagtgctataatgccgtgaagatgacaaaggacggcctgaccagagtgtacgtggacagggatggcgtgaacatcacagtgaatctgaagcctaccggaggactggcaaacggcgtgcggagatacgccagccagaccgagctgtatgatgcaccaggaagggtggaggcaacatacaggaccaggaccacagtgaactgtctgatcacagacatgatggccaagagcaattccccattcgatttctttgtgaccacaaccggccagaccgtggagatgagccccttttatgacggcaagaacacagagaccttccacgagcgcgccgattcctttcacgtgcggacaaattacaagatcgtggactatgataacagaggaaccaatccacagggagagaggagggccttcctggacaagggcacatacaccctgtcctggaagctggagaacaggacagcctattgccccctgcagcactggcagacatttgactccaccatcgccacagagaccggcaagtctatccacttcgtgacagatgagggcacctcctcttttgtgaccaacacaaccgtgggcatcgagctgcccgacgccttcaagtgtatcgaggagcaagtgaataagacaatgcacgagaagtacgaggccgtgcaggatcgctataccaagggccaggaagccatcacatactttatcaccagcggaggactgctgctggcatggctgccactgacaccacggtccctggccacagtgaagaatctgaccgagctgacaaccccaaccagctccccaccatctagcccaagccctccagcaccacctgcagcacggggctctaccagcgccgccgtgctgcggagaaggcgccggaacgcaggaaatgcaacaacccctgtgccaccagcagcacctggcaagtctctgggcacactgaacaatcccgccaccgtgcagatccagttcgcctacgacagcctgagaaggcagatcaacagaatgctgggcgatctggcaagggcatggtgcctggagcagaagcgccagaacatggtgctgcgggagctgaccaagatcaatcctacaaccgtgatgtcctctatctatggcaaggcagtggcagcaaagagactgggcgacgtgatctccgtgtctcagtgcgtgccagtgaatcaggccacagtgaccctgagaaagagcatgagggtgcccggctccgagaccatgtgctactctaggcctctggtgagcttctcctttatcaacgacacaaagacctatgagggccagctgggcacagataatgagatcttcctgacaaagaagatgaccgaggtgtgccaggccaccagccagtactatttccagtccggcaacgagatccacgtgtacaatgactatcaccactttaagacaatcgagctggatggcatcgccacactgcagaccttcatctctctgaacaccagcctgatcgagaatatcgactttgccagcctggagctgtactccagggacgagcagagggcatccaacgtgttcgatctggagggcatcttccgcgagtataactttcaggcccagaatatcgccggcctgcggaaggacctggataatgccgtgtctcaccaccaccaccaccac

SEQ ID NO: 3 - protein, 467 aa, synthetic construct
MGWSCIILFLVATATGVHSQVQLQQPGAELVRPGASVKLSCKASGFTFTSYWINWVKQRPGQGLEWIGNIFPSDSYTNYNQKFKDKATLTVDKSSSTAYMLLSSPTSEDSAVYYCTRGGYRYDSDYWGQGTTLTVSSASTKGPSVFPLAPSSKSTSGGTAALGCLVKDYFPEPVTVSWNSGALTSGVHTFPAVLQSSGLYSLSSVVTVPSSSLGTQTYICNVNHKPSNTKVDKRVEPKSCDKTHTCPPCPAPELLGGPSVFLFPPKPKDTLMISRTPEVTCVVVDVSHEDPEVKFNWYVDGVEVHNAKTKPREEQYNSTYRVVSVLTVLHQDWLNGKEYKCKVSNKALPAPIEKTISKAKGQPREPQVYTLPPSREEMTKNQVSLTCLVKGFYPSDIAVEWESNGQPENNYKTTPPVLDSDGSFFLYSKLTVDKSRWQQGNVFSCSVMHEALHNHYTQKSLSLSPGK

SEQ ID NO: 4 - protein, 118 aa, synthetic construct
QVQLQQPGAELVRPGASVKLSCKASGFTFTSYWINWVKQRPGQGLEWIGNIFPSDSYTNYNQKFKDKATLTVDKSSSTAYMLLSSPTSEDSAVYYCTRGGYRYDSDYWGQGTTLTVSS

SEQ ID NO: 5 - protein, 8 aa, synthetic construct
GFTFTSYW

SEQ ID NO: 6 - protein, 8 aa, synthetic construct
IFPSDSYT

SEQ ID NO: 7 - protein, 11 aa, synthetic construct
TRGGYRYDSDY

SEQ ID NO: 8 - protein, 5 aa, synthetic construct
SYWIN

SEQ ID NO: 9 - protein, 17 aa, synthetic construct
NIFPSDSYTNYNQKFKD

SEQ ID NO: 10 - protein, 9 aa, synthetic construct
GGYRYDSDY

SEQ ID NO: 11 - protein, 7 aa, synthetic construct
GFTFTSY

SEQ ID NO: 12 - protein, 6 aa, synthetic construct
FPSDSY

SEQ ID NO: 13 - protein, 6 aa, synthetic construct
TSYWIN

SEQ ID NO: 14 - protein, 13 aa, synthetic construct
WIGNIFPSDSYTN

SEQ ID NO: 15 - protein, 10 aa, synthetic construct
TRGGYRYDSD

SEQ ID NO: 16 - protein, 232 aa, synthetic construct
MGWSCIILFLVATATGSWAQIVLTQSPAIMSASPGEKVTMTCSASSSVTYMYWYQQKPGSSPRLLIYDTSNLASGVPVRFSGSGSGTSYSLTISRMEAEDAATYYCQQWSSYPYTFGGGTKLEIKRTVAAPSVFIFPPSDEQLKSGTASVVCLLNNFYPREAKVQWKVDNALQSGNSQESVTEQDSKDSTYSLSSTLTLSKADYEKHKVYACEVTHQGLSSPVTKSFNRGEC

SEQ ID NO: 17 - protein, 102 aa, synthetic construct
QIVLTQSPAIMSASPGEKVTMTCSASSSVTYMYWYQQKPGSSPRLLIYDTSNLASGVPVRFSGSGSGTSYSLTISRMEAEDAATYYCQQWSSYPYTFGGGTK

SEQ ID NO: 18 - protein, 5 aa, synthetic construct
SSVTY

SEQ ID NO: 19 - protein, 9 aa, synthetic construct
QQWSSYPYT

SEQ ID NO: 20 - protein, 10 aa, synthetic construct
SASSSVTYMY

SEQ ID NO: 21 - protein, 7 aa, synthetic construct
DTSNLAS

SEQ ID NO: 22 - protein, 6 aa, synthetic construct
TYMYWY

SEQ ID NO: 23 - protein, 10 aa, synthetic construct
LLIYDTSNLA

SEQ ID NO: 24 - protein, 8 aa, synthetic construct
QQWSSYPY

SEQ ID NO: 25 - protein, 4 aa, synthetic construct
GGGS